European Patent Application EP 4 656 204 A2, published December 3, 2025. Title: Anti-Axl Antibodies, Their Immunoconjugates and Uses Thereof. Applicant: BioAtla Inc. The sequence listing filed with the application follows.

SEQUENCE LISTING (116 sequences)

SEQ ID NO: 1 - skipped

SEQ ID NO: 2 - protein, 17 aa, synthetic construct
  REGION 1..17: note = Synthetic sequence
  SITE 4: note = Variants - It is P or N
  SITE 10: note = Variants - It is S or I or T
LIKXSNGGTXYNQKFKG

SEQ ID NO: 3 - skipped

SEQ ID NO: 4 - protein, 11 aa, synthetic construct
  REGION 1..11: note = Synthetic sequence
  SITE 6: note = Variants - It is V or D or G or N or W
  SITE 7: note = Variants - It is S or V
  SITE 9: note = Variants - It is A or L or M
  SITE 11: note = Variants - It is A or D or N or Q
KASQDXXSXVX

SEQ ID NO: 5-6 - skipped (2 entries)

SEQ ID NO: 7 - DNA, 323 bp, synthetic construct
  misc_feature 1..323: note = Synthetic sequence
  source 1..323: mol_type = other DNA
gacatccagatgacccagtctccatcctccctgtctgcatctgtaggagacagagtcaccatcacttgcaaggccagtcaggatgtggtttctgctgtagcctggtaccagcagaaacctggccaggctcccaggctcctcatctattggcaggatacccggcacactggagtcccatcaaggttcagcggcagtggatctgggacagaattcactctcaccatcagcagcctgcagcctgatgattttgcaacttattactgtcaggaacattttagcactccgctcacgttcggccaagggaccaaggtggaaatcaaacc

SEQ ID NO: 8 - DNA, 323 bp, synthetic construct
  misc_feature 1..323: note = Synthetic sequence
  source 1..323: mol_type = other DNA
gacatccagatgacccagtctccatcctccctgtctgcatctgtaggagacagagtcaccatcacttgcaaggccagtcaggatgtgagttctgctgtagcctggtaccagcagaaacctggccaggctcccaggctcctcatctattggcaggatacccggcacactggagtcccatcaaggttcagcggcagtggatctgggacagaattcactctcaccatcagcagcctgcagcctgatgattttgcaacttattactgtcaggaacattttagccctccgctcacgttcggccaagggaccaaggtggaaatcaaacc

SEQ ID NO: 9 - DNA, 323 bp, synthetic construct
  misc_feature 1..323: note = Synthetic sequence
  source 1..323: mol_type = other DNA
gacatccagatgacccagtctccatcctccctgtctgcatctgtaggagacagagtcaccatcacttgcaaggccagtcaggatgtggtttctgctgtagcctggtaccagcagaaacctggccaggctcccaggctcctcatctattggcaggatacccggcacactggagtcccatcaaggttcagcggcagtggatctgggacagaattcactctcaccatcagcagcctgcagcctgatgattttgcaacttattactgtcaggaacattttagccctccgctcacgttcggccaagggaccaaggtggaaatcaaacc

SEQ ID NO: 10 - DNA, 323 bp, synthetic construct
  misc_feature 1..323: note = Synthetic sequence
  source 1..323: mol_type = other DNA
gacatccagatgacccagtctccatcctccctgtctgcatctgtaggagacagagtcaccatcacttgcaaggccagtcaggatgtggtttctgctgtagcctggtaccagcagaaacctggccaggctcccaggctcctcatctattggcaggatacccggcacactggagtcccatcaaggttcagcggcagtggatctgggacagaattcactctcaccatcagcagcctgcagcctgatgattttgcaacttattactgtcaggaacattttagccctccgctcaggttcggccaagggaccaaggtggaaatcaaacc

SEQ ID NO: 11 - DNA, 360 bp, synthetic construct
  misc_feature 1..360: note = Synthetic sequence
  source 1..360: mol_type = other DNA
gaggtccagctggtacagtctggggctgaggtgaagaagcctggggctacagtgaaaatctcctgcaaggtttctggttactcattcactggcgctaccatgaactggatccgccagcccccagggaaggggctggagtggattggtcttattaaaccttccaatggtggtactagttacaaccagaagttcaagggcagagtcaccatctcagccgacaagtccatcagcaccgcctacctgcagtggagcagcctgaaggcctcggacaccgccatgtattactgtgcacatggtcactacgagagttacgaggctatggactactggggccagggaacgctggtcaccgtcagctca

SEQ ID NO: 12 - DNA, 360 bp, synthetic construct
  misc_feature 1..360: note = Synthetic sequence
  source 1..360: mol_type = other DNA
gaggtccagctggtacagtctggggctgaggtgaagaagcctggggctacagtgaaaatctcctgcaaggtttctggttactcattctggggcgctaccatgaactggatccgccagcccccagggaaggggctggagtggattggtcttattaaaccttccaatggtggtactagttacaaccagaagttcaagggcagagtcaccatctcagccgacaagtccatcagcaccgcctacctgcagtggagcagcctgaaggcctcggacaccgccatgtattactgtgcacatggtcactacgagagttacgaggctatggactactggggccagggaacgctggtcaccgtcagctca

SEQ ID NO: 13 - DNA, 360 bp, synthetic construct
  misc_feature 1..360: note = Synthetic sequence
  source 1..360: mol_type = other DNA
gaggtccagctggtacagtctggggctgaggtgaagaagcctggggctacagtgaaaatctcctgcaaggtttctggttactcattcactggccacaccatgaactggatccgccagcccccagggaaggggctggagtggattggtcttattaaaccttccaatggtggtactagttacaaccagaagttcaagggcagagtcaccatctcagccgacaagtccatcagcaccgcctacctgcagtggagcagcctgaaggcctcggacaccgccatgtattactgtgcacatggtcactacgagagttacgaggctatggactactggggccagggaacgctggtcaccgtcagctca

SEQ ID NO: 14 - protein, 120 aa, synthetic construct
  REGION 1..120: note = Synthetic sequence
EVQLVQSGAEVKKPGATVKISCKVSGYSFTGHTMNWIRQPPGKGLEWIGLIKPSNGGTSYNQKFKGRVTISADKSISTAYLQWSSLKASDTAMYYCAHGHYESYFAMDYWGQGTLVTVSS

SEQ ID NO: 15 - protein, 120 aa, synthetic construct
  REGION 1..120: note = Synthetic sequences
EVQLVQSGAEVKKPGATVKISCKVSGYSFAGHTMNWIRQPPGKGLEWIGLIKPSNGGTSYNQKFKGRVTISADKSISTAYLQWSSLKASDTAMYYCAHGHYESYFAMDYWGQGTLVTVSS

SEQ ID NO: 16 - protein, 120 aa, synthetic construct
  REGION 1..120: note = Synthetic sequence
EVQLVQSGAEVKKPGATVKISCKVSGYSFWGHTMNWIRQPPGKGLEWIGLIKPSNGGTSYNQKFKGRVTISADKSISTAYLQWSSLKASDTAMYYCAHGHYESYFAMDYWGQGTLVTVSS

SEQ ID NO: 17 - protein, 120 aa, synthetic construct
  REGION 1..120: note = Synthetic sequence
EVQLVQSGAEVKKPGATVKISCKVSGYSFTGATMNWIRQPPGKGLEWIGLIKPSNGGTSYNQKFKGRVTISADKSISTAYLQWSSLKASDTAMYYCAHGHYESYFAMDYWGQGTLVTVSS

SEQ ID NO: 18 - protein, 120 aa, synthetic construct
  REGION 1..120: note = Synthetic sequence
EVQLVQSGAEVKKPGATVKISCKVSGYSFTGHIMNWIRQPPGKGLEWIGLIKPSNGGTSYNQKFKGRVTISADKSISTAYLQWSSLKASDTAMYYCAHGHYESYFAMDYWGQGTLVTVSS

SEQ ID NO: 19 - protein, 120 aa, synthetic construct
  REGION 1..120: note = Synthetic sequence
EVQLVQSGAEVKKPGATVKISCKVSGYSFTGHTMIWIRQPPGKGLEWIGLIKPSNGGTSYNQKFKGRVTISADKSISTAYLQWSSLKASDTAMYYCAHGHYESYFAMDYWGQGTLVTVSS

SEQ ID NO: 20 - protein, 120 aa, synthetic construct
  REGION 1..120: note = Synthetic sequence
EVQLVQSGAEVKKPGATVKISCKVSGYSFTGHTMNWIRQPPGKGLEWIGLIKNSNGGTSYNQKFKGRVTISADKSISTAYLQWSSLKASDTAMYYCAHGHYESYFAMDYWGQGTLVTVSS

SEQ ID NO: 21 - protein, 120 aa, synthetic construct
  REGION 1..120: note = Synthetic sequences
EVQLVQSGAEVKKPGATVKISCKVSGYSFTGHTMNWIRQPPGKGLEWIGLIKPSNGGTIYNQKFKGRVTISADKSISTAYLQWSSLKASDTAMYYCAHGHYESYFAMDYWGQGTLVTVSS

SEQ ID NO: 22 - protein, 120 aa, synthetic construct
  REGION 1..120: note = Synthetic sequence
EVQLVQSGAEVKKPGATVKISCKVSGYSFTGHTMNWIRQPPGKGLEWIGLIKPSNGGTTYNQKFKGRVTISADKSISTAYLQWSSLKASDTAMYYCAHGHYESYFAMDYWGQGTLVTVSS

SEQ ID NO: 23 - protein, 120 aa, synthetic construct
  REGION 1..120: note = Synthetic sequence
EVQLVQSGAEVKKPGATVKISCKVSGYSFTGHTMNWIRQPPGKGLEWIGLIKPSNGGTSYNQKFKGRVTISADKSISTAYLQWSSLKASDTAMYYCAHGRYESYFAMDYWGQGTLVTVSS

SEQ ID NO: 24 - protein, 120 aa, synthetic construct
  REGION 1..120: note = Synthetic sequence
EVQLVQSGAEVKKPGATVKISCKVSGYSFTGHTMNWIRQPPGKGLEWIGLIKPSNGGTSYNQKFKGRVTISADKSISTAYLQWSSLKASDTAMYYCAHGDYESYFAMDYWGQGTLVTVSS

SEQ ID NO: 25 - protein, 120 aa, synthetic construct
  REGION 1..120: note = Synthetic sequence
EVQLVQSGAEVKKPGATVKISCKVSGYSFTGHTMNWIRQPPGKGLEWIGLIKPSNGGTSYNQKFKGRVTISADKSISTAYLQWSSLKASDTAMYYCAHGEYESYFAMDYWGQGTLVTVSS

SEQ ID NO: 26 - protein, 120 aa, synthetic construct
  REGION 1..120: note = Synthetic sequence
EVQLVQSGAEVKKPGATVKISCKVSGYSFTGHTMNWIRQPPGKGLEWIGLIKPSNGGTSYNQKFKGRVTISADKSISTAYLQWSSLKASDTAMYYCAHGWYESYFAMDYWGQGTLVTVSS

SEQ ID NO: 27 - protein, 120 aa, synthetic construct
  REGION 1..120: note = Synthetic sequence
EVQLVQSGAEVKKPGATVKISCKVSGYSFTGHTMNWIRQPPGKGLEWIGLIKPSNGGTSYNQKFKGRVTISADKSISTAYLQWSSLKASDTAMYYCAHGPYESYFAMDYWGQGTLVTVSS

SEQ ID NO: 28 - protein, 120 aa, synthetic construct
  REGION 1..120: note = Synthetic sequence
EVQLVQSGAEVKKPGATVKISCKVSGYSFTGHTMNWIRQPPGKGLEWIGLIKPSNGGTSYNQKFKGRVTISADKSISTAYLQWSSLKASDTAMYYCAHGHNESYFAMDYWGQGTLVTVSS

SEQ ID NO: 29 - protein, 120 aa, synthetic construct
  REGION 1..120: note = Synthetic sequence
EVQLVQSGAEVKKPGATVKISCKVSGYSFTGHTMNWIRQPPGKGLEWIGLIKPSNGGTSYNQKFKGRVTISADKSISTAYLQWSSLKASDTAMYYCAHGHYFSYFAMDYWGQGTLVTVSS

SEQ ID NO: 30 - protein, 120 aa, synthetic construct
  REGION 1..120: note = Synthetic sequence
EVQLVQSGAEVKKPGATVKISCKVSGYSFTGHTMNWIRQPPGKGLEWIGLIKPSNGGTSYNQKFKGRVTISADKSISTAYLQWSSLKASDTAMYYCAHGHYISYFAMDYWGQGTLVTVSS

SEQ ID NO: 31 - protein, 120 aa, synthetic construct
  REGION 1..120: note = Synthetic sequence
EVQLVQSGAEVKKPGATVKISCKVSGYSFTGHTMNWIRQPPGKGLEWIGLIKPSNGGTSYNQKFKGRVTISADKSISTAYLQWSSLKASDTAMYYCAHGHYASYFAMDYWGQGTLVTVSS

SEQ ID NO: 32 - protein, 120 aa, synthetic construct
  REGION 1..120: note = Synthetic sequence
EVQLVQSGAEVKKPGATVKISCKVSGYSFTGHTMNWIRQPPGKGLEWIGLIKPSNGGTSYNQKFKGRVTISADKSISTAYLQWSSLKASDTAMYYCAHGHYDSYFAMDYWGQGTLVTVSS

SEQ ID NO: 33 - protein, 120 aa, synthetic construct
  REGION 1..120: note = Synthetic sequence
EVQLVQSGAEVKKPGATVKISCKVSGYSFTGHTMNWIRQPPGKGLEWIGLIKPSNGGTSYNQKFKGRVTISADKSISTAYLQWSSLKASDTAMYYCAHGHYGSYFAMDYWGQGTLVTVSS

SEQ ID NO: 34 - protein, 120 aa, synthetic construct
  REGION 1..120: note = Synthetic sequence
EVQLVQSGAEVKKPGATVKISCKVSGYSFTGHTMNWIRQPPGKGLEWIGLIKPSNGGTSYNQKFKGRVTISADKSISTAYLQWSSLKASDTAMYYCAHGHYHSYFAMDYWGQGTLVTVSS

SEQ ID NO: 35 - protein, 120 aa, synthetic construct
  REGION 1..120: note = Synthetic sequence
EVQLVQSGAEVKKPGATVKISCKVSGYSFTGHTMNWIRQPPGKGLEWIGLIKPSNGGTSYNQKFKGRVTISADKSISTAYLQWSSLKASDTAMYYCAHGHYLSYFAMDYWGQGTLVTVSS

SEQ ID NO: 36 - protein, 120 aa, synthetic construct
  REGION 1..120: note = Synthetic sequence
EVQLVQSGAEVKKPGATVKISCKVSGYSFTGHTMNWIRQPPGKGLEWIGLIKPSNGGTSYNQKFKGRVTISADKSISTAYLQWSSLKASDTAMYYCAHGHYMSYFAMDYWGQGTLVTVSS

SEQ ID NO: 37 - protein, 120 aa, synthetic construct
  REGION 1..120: note = Synthetic sequence
EVQLVQSGAEVKKPGATVKISCKVSGYSFTGHTMNWIRQPPGKGLEWIGLIKPSNGGTSYNQKFKGRVTISADKSISTAYLQWSSLKASDTAMYYCAHGHYNSYFAMDYWGQGTLVTVSS

SEQ ID NO: 38 - protein, 120 aa, synthetic construct
  REGION 1..120: note = Synthetic sequence
EVQLVQSGAEVKKPGATVKISCKVSGYSFTGHTMNWIRQPPGKGLEWIGLIKPSNGGTSYNQKFKGRVTISADKSISTAYLQWSSLKASDTAMYYCAHGHYRSYFAMDYWGQGTLVTVSS

SEQ ID NO: 39 - protein, 120 aa, synthetic construct
  REGION 1..120: note = Synthetic sequence
EVQLVQSGAEVKKPGATVKISCKVSGYSFTGHTMNWIRQPPGKGLEWIGLIKPSNGGTSYNQKFKGRVTISADKSISTAYLQWSSLKASDTAMYYCAHGHYVSYFAMDYWGQGTLVTVSS

SEQ ID NO: 40 - protein, 120 aa, synthetic construct
  REGION 1..120: note = Synthetic sequence
EVQLVQSGAEVKKPGATVKISCKVSGYSFTGHTMNWIRQPPGKGLEWIGLIKPSNGGTSYNQKFKGRVTISADKSISTAYLQWSSLKASDTAMYYCAHGHYYSYFAMDYWGQGTLVTVSS

SEQ ID NO: 41 - protein, 120 aa, synthetic construct
  REGION 1..120: note = Synthetic sequence
EVQLVQSGAEVKKPGATVKISCKVSGYSFTGHTMNWIRQPPGKGLEWIGLIKPSNGGTSYNQKFKGRVTISADKSISTAYLQWSSLKASDTAMYYCAHGHYEDYFAMDYWGQGTLVTVSS

SEQ ID NO: 42 - protein, 120 aa, synthetic construct
  REGION 1..120: note = Synthetic sequence
EVQLVQSGAEVKKPGATVKISCKVSGYSFTGHTMNWIRQPPGKGLEWIGLIKPSNGGTSYNQKFKGRVTISADKSISTAYLQWSSLKASDTAMYYCAHGHYEMYFAMDYWGQGTLVTVSS

SEQ ID NO: 43 - protein, 120 aa, synthetic construct
  REGION 1..120: note = Synthetic sequence
EVQLVQSGAEVKKPGATVKISCKVSGYSFTGHTMNWIRQPPGKGLEWIGLIKPSNGGTSYNQKFKGRVTISADKSISTAYLQWSSLKASDTAMYYCAHGHYENYFAMDYWGQGTLVTVSS

SEQ ID NO: 44 - protein, 120 aa, synthetic construct
  REGION 1..120: note = Synthetic sequence
EVQLVQSGAEVKKPGATVKISCKVSGYSFTGHTMNWIRQPPGKGLEWIGLIKPSNGGTSYNQKFKGRVTISADKSISTAYLQWSSLKASDTAMYYCAHGHYEQYFAMDYWGQGTLVTVSS

SEQ ID NO: 45 - protein, 120 aa, synthetic construct
  REGION 1..120: note = Synthetic sequence
EVQLVQSGAEVKKPGATVKISCKVSGYSFTGHTMNWIRQPPGKGLEWIGLIKPSNGGTSYNQKFKGRVTISADKSISTAYLQWSSLKASDTAMYYCAHGHYESCFAMDYWGQGTLVTVSS

SEQ ID NO: 46 - protein, 120 aa, synthetic construct
  REGION 1..120: note = Synthetic sequence
EVQLVQSGAEVKKPGATVKISCKVSGYSFTGHTMNWIRQPPGKGLEWIGLIKPSNGGTSYNQKFKGRVTISADKSISTAYLQWSSLKASDTAMYYCAHGHYESEFAMDYWGQGTLVTVSS

SEQ ID NO: 47 - protein, 120 aa, synthetic construct
  REGION 1..120: note = Synthetic sequence
EVQLVQSGAEVKKPGATVKISCKVSGYSFTGHTMNWIRQPPGKGLEWIGLIKPSNGGTSYNQKFKGRVTISADKSISTAYLQWSSLKASDTAMYYCAHGHYESPFAMDYWGQGTLVTVSS

SEQ ID NO: 48 - protein, 120 aa, synthetic construct
  REGION 1..120: note = Synthetic sequence
EVQLVQSGAEVKKPGATVKISCKVSGYSFTGHTMNWIRQPPGKGLEWIGLIKPSNGGTSYNQKFKGRVTISADKSISTAYLQWSSLKASDTAMYYCAHGHYESYEAMDYWGQGTLVTVSS

SEQ ID NO: 49 - protein, 120 aa, synthetic construct
  REGION 1..120: note = Synthetic sequence
EVQLVQSGAEVKKPGATVKISCKVSGYSFTGHTMNWIRQPPGKGLEWIGLIKPSNGGTSYNQKFKGRVTISADKSISTAYLQWSSLKASDTAMYYCAHGHYESYNAMDYWGQGTLVTVSS

SEQ ID NO: 50 - protein, 120 aa, synthetic construct
  REGION 1..120: note = Synthetic sequence
EVQLVQSGAEVKKPGATVKISCKVSGYSFTGHTMNWIRQPPGKGLEWIGLIKPSNGGTSYNQKFKGRVTISADKSISTAYLQWSSLKASDTAMYYCAHGHYESYSAMDYWGQGTLVTVSS

SEQ ID NO: 51 - protein, 120 aa, synthetic construct
  REGION 1..120: note = Synthetic sequence
EVQLVQSGAEVKKPGATVKISCKVSGYSFTGHTMNWIRQPPGKGLEWIGLIKPSNGGTSYNQKFKGRVTISADKSISTAYLQWSSLKASDTAMYYCAHGHYESYTAMDYWGQGTLVTVSS

SEQ ID NO: 52 - protein, 120 aa, synthetic construct
  REGION 1..120: note = Synthetic sequence
EVQLVQSGAEVKKPGATVKISCKVSGYSFTGHTMNWIRQPPGKGLEWIGLIKPSNGGTSYNQKFKGRVTISADKSISTAYLQWSSLKASDTAMYYCAHGHYESYVAMDYWGQGTLVTVSS

SEQ ID NO: 53 - protein, 120 aa, synthetic construct
  REGION 1..120: note = Synthetic sequence
EVQLVQSGAEVKKPGATVKISCKVSGYSFTGHTMNWIRQPPGKGLEWIGLIKPSNGGTSYNQKFKGRVTISADKSISTAYLQWSSLKASDTAMYYCAHGHYESYFDMDYWGQGTLVTVSS

SEQ ID NO: 54 - protein, 120 aa, synthetic construct
  REGION 1..120: note = Synthetic sequence
EVQLVQSGAEVKKPGATVKISCKVSGYSFTGHTMNWIRQPPGKGLEWIGLIKPSNGGTSYNQKFKGRVTISADKSISTAYLQWSSLKASDTAMYYCAHGHYESYFGMDYWGQGTLVTVSS

SEQ ID NO: 55 - protein, 120 aa, synthetic construct
  REGION 1..120: note = Synthetic sequence
EVQLVQSGAEVKKPGATVKISCKVSGYSFTGHTMNWIRQPPGKGLEWIGLIKPSNGGTSYNQKFKGRVTISADKSISTAYLQWSSLKASDTAMYYCAHGHYESYFLMDYWGQGTLVTVSS

SEQ ID NO: 56 - protein, 120 aa, synthetic construct
  REGION 1..120: note = Synthetic sequence
EVQLVQSGAEVKKPGATVKISCKVSGYSFTGHTMNWIRQPPGKGLEWIGLIKPSNGGTSYNQKFKGRVTISADKSISTAYLQWSSLKASDTAMYYCAHGHYESYFYMDYWGQGTLVTVSS

SEQ ID NO: 57 - protein, 120 aa, synthetic construct
  REGION 1..120: note = Synthetic sequence
EVQLVQSGAEVKKPGATVKISCKVSGYSFTGHTMNWIRQPPGKGLEWIGLIKPSNGGTSYNQKFKGRVTISADKSISTAYLQWSSLKASDTAMYYCAHGHYESYFAEDYWGQGTLVTVSS

SEQ ID NO: 58 - protein, 120 aa, synthetic construct
  REGION 1..120: note = Synthetic sequence
EVQLVQSGAEVKKPGATVKISCKVSGYSFTGHTMNWIRQPPGKGLEWIGLIKPSNGGTSYNQKFKGRVTISADKSISTAYLQWSSLKASDTAMYYCAHGHYESYFAFDYWGQGTLVTVSS

SEQ ID NO: 59 - protein, 120 aa, synthetic construct
  REGION 1..120: note = Synthetic sequence
EVQLVQSGAEVKKPGATVKISCKVSGYSFTGHTMNWIRQPPGKGLEWIGLIKPSNGGTSYNQKFKGRVTISADKSISTAYLQWSSLKASDTAMYYCAHGHYESYFAMDYPGQGTLVTVSS

SEQ ID NO: 60 - protein, 120 aa, synthetic construct
  REGION 1..120: note = Synthetic sequence
EVQLVQSGAEVKKPGATVKISCKVSGYSFTGHTMNWIRQPPGKGLEWIGLIKPSNGGTSYNQKFKGRVTISADKSISTAYLQWSSLKASDTAMYYCAHGHYESYFAMDYHGQGTLVTVSS

SEQ ID NO: 61 - protein, 120 aa, synthetic construct
  REGION 1..120: note = Synthetic sequence
EVQLVQSGAEVKKPGATVKISCKVSGYSFTGHTMNWIRQPPGKGLEWIGLIKPSNGGTSYNQKFKGRVTISADKSISTAYLQWSSLKASDTAMYYCAHGHYESYFAMDYTGQGTLVTVSS

SEQ ID NO: 62 - protein, 120 aa, synthetic construct
  REGION 1..120: note = Synthetic sequence
EVQLVQSGAEVKKPGATVKISCKVSGYSFTGHTMNWIRQPPGKGLEWIGLIKPSNGGTSYNQKFKGRVTISADKSISTAYLQWSSLKASDTAMYYCAHGHYESYFAMDYNGQGTLVTVSS

SEQ ID NO: 63 - protein, 120 aa, synthetic construct
  REGION 1..120: note = Synthetic sequence
EVQLVQSGAEVKKPGATVKISCKVSGYSFTGHTMNWIRQPPGKGLEWIGLIKPSNGGTSYNQKFKGRVTISADKSISTAYLQWSSLKASDTAMYYCAHGHYESYFAMDYLGQGTLVTVSS

SEQ ID NO: 64 - protein, 120 aa, synthetic construct
  REGION 1..120: note = Synthetic sequence
EVQLVQSGAEVKKPGATVKISCKVSGYSFTGHTMNWIRQPPGKGLEWIGLIKPSNGGTSYNQKFKGRVTISADKSISTAYLQWSSLKASDTAMYYCAHGHYESYFAMDYRGQGTLVTVSS

SEQ ID NO: 65 - protein, 120 aa, synthetic construct
  REGION 1..120: note = Synthetic sequence
EVQLVQSGAEVKKPGATVKISCKVSGYSFTGHTMNWIRQPPGKGLEWIGLIKPSNGGTSYNQKFKGRVTISADKSISTAYLQWSSLKASDTAMYYCAHGHYESYFAMDYDGQGTLVTVSS

SEQ ID NO: 66 - protein, 120 aa, synthetic construct
  REGION 1..120: note = Synthetic sequence
EVQLVQSGAEVKKPGATVKISCKVSGYSFTGHTMNWIRQPPGKGLEWIGLIKPSNGGTSYNQKFKGRVTISADKSISTAYLQWSSLKASDTAMYYCAHGHYESYFAMDYAGQGTLVTVSS

SEQ ID NO: 67 - protein, 120 aa, synthetic construct
  REGION 1..120: note = Synthetic sequence
EVQLVQSGAEVKKPGATVKISCKVSGYSFTGHTMNWIRQPPGKGLEWIGLIKPSNGGTSYNQKFKGRVTISADKSISTAYLQWSSLKASDTAMYYCAHGHYESYFAMDYWHQGTLVTVSS

SEQ ID NO: 68 - protein, 107 aa, synthetic construct
  REGION 1..107: note = Synthetic sequence
DIQMTQSPSSLSASVGDRVTITCKASQDVSSAVAWYQQKPGQAPRLLIYWASTRHTGVPSRFSGSGSGTEFTLTISSLQPDDFATYYCQEHFSTPLTFGQGTKVEIK

SEQ ID NO: 69 - protein, 107 aa, synthetic construct
  REGION 1..107: note = Synthetic sequence
DIQMTQSPSSLSASVGDRVTITCKASQDDSSAVAWYQQKPGQAPRLLIYWASTRHTGVPSRFSGSGSGTEFTLTISSLQPDDFATYYCQEHFSTPLTFGQGTKVEIK

SEQ ID NO: 70 - protein, 107 aa, synthetic construct
  REGION 1..107: note = Synthetic sequence
DIQMTQSPSSLSASVGDRVTITCKASQDGSSAVAWYQQKPGQAPRLLIYWASTRHTGVPSRFSGSGSGTEFTLTISSLQPDDFATYYCQEHFSTPLTFGQGTKVEIK

SEQ ID NO: 71 - protein, 107 aa, synthetic construct
  REGION 1..107: note = Synthetic sequence
DIQMTQSPSSLSASVGDRVTITCKASQDNSSAVAWYQQKPGQAPRLLIYWASTRHTGVPSRFSGSGSGTEFTLTISSLQPDDFATYYCQEHFSTPLTFGQGTKVEIK

SEQ ID NO: 72 - protein, 107 aa, synthetic construct
  REGION 1..107: note = Synthetic sequence
DIQMTQSPSSLSASVGDRVTITCKASQDWSSAVAWYQQKPGQAPRLLIYWASTRHTGVPSRFSGSGSGTEFTLTISSLQPDDFATYYCQEHFSTPLTFGQGTKVEIK

SEQ ID NO: 73 - protein, 107 aa, synthetic construct
  REGION 1..107: note = Synthetic sequence
DIQMTQSPSSLSASVGDRVTITCKASQDVVSAVAWYQQKPGQAPRLLIYWASTRHTGVPSRFSGSGSGTEFTLTISSLQPDDFATYYCQEHFSTPLTFGQGTKVEIK

SEQ ID NO: 74 - protein, 107 aa, synthetic construct
  REGION 1..107: note = Synthetic sequence
DIQMTQSPSSLSASVGDRVTITCKASQDVSSLVAWYQQKPGQAPRLLIYWASTRHTGVPSRFSGSGSGTEFTLTISSLQPDDFATYYCQEHFSTPLTFGQGTKVEIK

SEQ ID NO: 75 - protein, 107 aa, synthetic construct
  REGION 1..107: note = Synthetic sequence
DIQMTQSPSSLSASVGDRVTITCKASQDVSSMVAWYQQKPGQAPRLLIYWASTRHTGVPSRFSGSGSGTEFTLTISSLQPDDFATYYCQEHFSTPLTFGQGTKVEIK

SEQ ID NO: 76 - protein, 107 aa, synthetic construct
  REGION 1..107: note = Synthetic sequence
DIQMTQSPSSLSASVGDRVTITCKASQDVSSAVDWYQQKPGQAPRLLIYWASTRHTGVPSRFSGSGSGTEFTLTISSLQPDDFATYYCQEHFSTPLTFGQGTKVEIK

SEQ ID NO: 77 - protein, 107 aa, synthetic construct
  REGION 1..107: note = Synthetic sequence
DIQMTQSPSSLSASVGDRVTITCKASQDVSSAVNWYQQKPGQAPRLLIYWASTRHTGVPSRFSGSGSGTEFTLTISSLQPDDFATYYCQEHFSTPLTFGQGTKVEIK

SEQ ID NO: 78 - protein, 107 aa, synthetic construct
  REGION 1..107: note = Synthetic sequence
DIQMTQSPSSLSASVGDRVTITCKASQDVSSAVQWYQQKPGQAPRLLIYWASTRHTGVPSRFSGSGSGTEFTLTISSLQPDDFATYYCQEHFSTPLTFGQGTKVEIK

SEQ ID NO: 79 - protein, 107 aa, synthetic construct
  REGION 1..107: note = Synthetic sequence
DIQMTQSPSSLSASVGDRVTITCKASQDVSSAVAWYQQKPGQAPRLLIYFASTRHTGVPSRFSGSGSGTEFTLTISSLQPDDFATYYCQEHFSTPLTFGQGTKVEIK

SEQ ID NO: 80 - protein, 107 aa, synthetic construct
  REGION 1..107: note = Synthetic sequence
DIQMTQSPSSLSASVGDRVTITCKASQDVSSAVAWYQQKPGQAPRLLIYWISTRHTGVPSRFSGSGSGTEFTLTISSLQPDDFATYYCQEHFSTPLTFGQGTKVEIK

SEQ ID NO: 81 - protein, 107 aa, synthetic construct
  REGION 1..107: note = Synthetic sequence
DIQMTQSPSSLSASVGDRVTITCKASQDVSSAVAWYQQKPGQAPRLLIYWNSTRHTGVPSRFSGSGSGTEFTLTISSLQPDDFATYYCQEHFSTPLTFGQGTKVEIK

SEQ ID NO: 82 - protein, 107 aa, synthetic construct
  REGION 1..107: note = Synthetic sequence
DIQMTQSPSSLSASVGDRVTITCKASQDVSSAVAWYQQKPGQAPRLLIYWPSTRHTGVPSRFSGSGSGTEFTLTISSLQPDDFATYYCQEHFSTPLTFGQGTKVEIK

SEQ ID NO: 83 - protein, 107 aa, synthetic construct
  REGION 1..107: note = Synthetic sequence
DIQMTQSPSSLSASVGDRVTITCKASQDVSSAVAWYQQKPGQAPRLLIYWQSTRHTGVPSRFSGSGSGTEFTLTISSLQPDDFATYYCQEHFSTPLTFGQGTKVEIK

SEQ ID NO: 84 - protein, 107 aa, synthetic construct
  REGION 1..107: note = Synthetic sequence
DIQMTQSPSSLSASVGDRVTITCKASQDVSSAVAWYQQKPGQAPRLLIYWADTRHTGVPSRFSGSGSGTEFTLTISSLQPDDFATYYCQEHFSTPLTFGQGTKVEIK

SEQ ID NO: 85 - protein, 107 aa, synthetic construct
  REGION 1..107: note = Synthetic sequence
DIQMTQSPSSLSASVGDRVTITCKASQDVSSAVAWYQQKPGQAPRLLIYWASTRDTGVPSRFSGSGSGTEFTLTISSLQPDDFATYYCQEHFSTPLTFGQGTKVEIK

SEQ ID NO: 86 - protein, 107 aa, synthetic construct
  REGION 1..107: note = Synthetic sequence
DIQMTQSPSSLSASVGDRVTITCKASQDVSSAVAWYQQKPGQAPRLLIYWASTRHTGVPSRFSGSGSGTEFTLTISSLQPDDFATYYCQECFSTPLTFGQGTKVEIK

SEQ ID NO: 87 - protein, 107 aa, synthetic construct
  REGION 1..107: note = Synthetic sequence
DIQMTQSPSSLSASVGDRVTITCKASQDVSSAVAWYQQKPGQAPRLLIYWASTRHTGVPSRFSGSGSGTEFTLTISSLQPDDFATYYCQEFFSTPLTFGQGTKVEIK

SEQ ID NO: 88 - protein, 107 aa, synthetic construct
  REGION 1..107: note = Synthetic sequence
DIQMTQSPSSLSASVGDRVTITCKASQDVSSAVAWYQQKPGQAPRLLIYWASTRHTGVPSRFSGSGSGTEFTLTISSLQPDDFATYYCQEIFSTPLTFGQGTKVEIK

SEQ ID NO: 89 - protein, 107 aa, synthetic construct
  REGION 1..107: note = Synthetic sequence
DIQMTQSPSSLSASVGDRVTITCKASQDVSSAVAWYQQKPGQAPRLLIYWASTRHTGVPSRFSGSGSGTEFTLTISSLQPDDFATYYCQELFSTPLTFGQGTKVEIK

SEQ ID NO: 90 - protein, 107 aa, synthetic construct
  REGION 1..107: note = Synthetic sequence
DIQMTQSPSSLSASVGDRVTITCKASQDVSSAVAWYQQKPGQAPRLLIYWASTRHTGVPSRFSGSGSGTEFTLTISSLQPDDFATYYCQEQFSTPLTFGQGTKVEIK

SEQ ID NO: 91 - protein, 107 aa, synthetic construct
  REGION 1..107: note = Synthetic sequence
DIQMTQSPSSLSASVGDRVTITCKASQDVSSAVAWYQQKPGQAPRLLIYWASTRHTGVPSRFSGSGSGTEFTLTISSLQPDDFATYYCQESFSTPLTFGQGTKVEIK

SEQ ID NO: 92 - protein, 107 aa, synthetic construct
  REGION 1..107: note = Synthetic sequence
DIQMTQSPSSLSASVGDRVTITCKASQDVSSAVAWYQQKPGQAPRLLIYWASTRHTGVPSRFSGSGSGTEFTLTISSLQPDDFATYYCQETFSTPLTFGQGTKVEIK

SEQ ID NO: 93 - protein, 107 aa, synthetic construct
  REGION 1..107: note = Synthetic sequence
DIQMTQSPSSLSASVGDRVTITCKASQDVSSAVAWYQQKPGQAPRLLIYWASTRHTGVPSRFSGSGSGTEFTLTISSLQPDDFATYYCQEVFSTPLTFGQGTKVEIK

SEQ ID NO: 94 - protein, 107 aa, synthetic construct
  REGION 1..107: note = Synthetic sequence
DIQMTQSPSSLSASVGDRVTITCKASQDVSSAVAWYQQKPGQAPRLLIYWASTRHTGVPSRFSGSGSGTEFTLTISSLQPDDFATYYCQEYFSTPLTFGQGTKVEIK

SEQ ID NO: 95 - protein, 107 aa, synthetic construct
  REGION 1..107: note = Synthetic sequence
DIQMTQSPSSLSASVGDRVTITCKASQDVSSAVAWYQQKPGQAPRLLIYWASTRHTGVPSRFSGSGSGTEFTLTISSLQPDDFATYYCQEHCSTPLTFGQGTKVEIK

SEQ ID NO: 96 - protein, 107 aa, synthetic construct
  REGION 1..107: note = Synthetic sequence
DIQMTQSPSSLSASVGDRVTITCKASQDVSSAVAWYQQKPGQAPRLLIYWASTRHTGVPSRFSGSGSGTEFTLTISSLQPDDFATYYCQEHDSTPLTFGQGTKVEIK

SEQ ID NO: 97 - protein, 107 aa, synthetic construct
  REGION 1..107: note = Synthetic sequence
DIQMTQSPSSLSASVGDRVTITCKASQDVSSAVAWYQQKPGQAPRLLIYWASTRHTGVPSRFSGSGSGTEFTLTISSLQPDDFATYYCQEHESTPLTFGQGTKVEIK

SEQ ID NO: 98 - protein, 107 aa, synthetic construct
  REGION 1..107: note = Synthetic sequence
DIQMTQSPSSLSASVGDRVTITCKASQDVSSAVAWYQQKPGQAPRLLIYWASTRHTGVPSRFSGSGSGTEFTLTISSLQPDDFATYYCQEHGSTPLTFGQGTKVEIK

SEQ ID NO: 99 - protein, 107 aa, synthetic construct
  REGION 1..107: note = Synthetic sequence
DIQMTQSPSSLSASVGDRVTITCKASQDVSSAVAWYQQKPGQAPRLLIYWASTRHTGVPSRFSGSGSGTEFTLTISSLQPDDFATYYCQEHNSTPLTFGQGTKVEIK

SEQ ID NO: 100 - protein, 107 aa, synthetic construct
  REGION 1..107: note = Synthetic sequence
DIQMTQSPSSLSASVGDRVTITCKASQDVSSAVAWYQQKPGQAPRLLIYWASTRHTGVPSRFSGSGSGTEFTLTISSLQPDDFATYYCQEHSSTPLTFGQGTKVEIK

SEQ ID NO: 101 - protein, 107 aa, synthetic construct
  REGION 1..107: note = Synthetic sequence
DIQMTQSPSSLSASVGDRVTITCKASQDVSSAVAWYQQKPGQAPRLLIYWASTRHTGVPSRFSGSGSGTEFTLTISSLQPDDFATYYCQEHFSCPLTFGQGTKVEIK

SEQ ID NO: 102 - protein, 107 aa, synthetic construct
  REGION 1..107: note = Synthetic sequence
DIQMTQSPSSLSASVGDRVTITCKASQDVSSAVAWYQQKPGQAPRLLIYWASTRHTGVPSRFSGSGSGTEFTLTISSLQPDDFATYYCQEHFSPPLTFGQGTKVEIK

SEQ ID NO: 103 - protein, 107 aa, synthetic construct
  REGION 1..107: note = Synthetic sequence
DIQMTQSPSSLSASVGDRVTITCKASQDVSSAVAWYQQKPGQAPRLLIYWASTRHTGVPSRFSGSGSGTEFTLTISSLQPDDFATYYCQEHFSTALTFGQGTKVEIK

SEQ ID NO: 104 - protein, 107 aa, synthetic construct
  REGION 1..107: note = Synthetic sequence
DIQMTQSPSSLSASVGDRVTITCKASQDVSSAVAWYQQKPGQAPRLLIYWASTRHTGVPSRFSGSGSGTEFTLTISSLQPDDFATYYCQEHFSTCLTFGQGTKVEIK

SEQ ID NO: 105 - protein, 107 aa, synthetic construct
  REGION 1..107: note = Synthetic sequence
DIQMTQSPSSLSASVGDRVTITCKASQDVSSAVAWYQQKPGQAPRLLIYWASTRHTGVPSRFSGSGSGTEFTLTISSLQPDDFATYYCQEHFSTDLTFGQGTKVEIK

SEQ ID NO: 106 - protein, 107 aa, synthetic construct
  REGION 1..107: note = Synthetic sequence
DIQMTQSPSSLSASVGDRVTITCKASQDVSSAVAWYQQKPGQAPRLLIYWASTRHTGVPSRFSGSGSGTEFTLTISSLQPDDFATYYCQEHFSTELTFGQGTKVEIK

SEQ ID NO: 107 - protein, 107 aa, synthetic construct
  REGION 1..107: note = Synthetic sequence
DIQMTQSPSSLSASVGDRVTITCKASQDVSSAVAWYQQKPGQAPRLLIYWASTRHTGVPSRFSGSGSGTEFTLTISSLQPDDFATYYCQEHFSTHLTFGQGTKVEIK

SEQ ID NO: 108 - protein, 107 aa, synthetic construct
  REGION 1..107: note = Synthetic sequence
DIQMTQSPSSLSASVGDRVTITCKASQDVSSAVAWYQQKPGQAPRLLIYWASTRHTGVPSRFSGSGSGTEFTLTISSLQPDDFATYYCQEHFSTKLTFGQGTKVEIK

SEQ ID NO: 109 - protein, 107 aa, synthetic construct
  REGION 1..107: note = Synthetic sequence
DIQMTQSPSSLSASVGDRVTITCKASQDVSSAVAWYQQKPGQAPRLLIYWASTRHTGVPSRFSGSGSGTEFTLTISSLQPDDFATYYCQEHFSTSLTFGQGTKVEIK

SEQ ID NO: 110 - protein, 107 aa, synthetic construct
  REGION 1..107: note = Synthetic sequence
DIQMTQSPSSLSASVGDRVTITCKASQDVSSAVAWYQQKPGQAPRLLIYWASTRHTGVPSRFSGSGSGTEFTLTISSLQPDDFATYYCQEHFSTTLTFGQGTKVEIK

SEQ ID NO: 111 - protein, 107 aa, synthetic construct
  REGION 1..107: note = Synthetic sequence
DIQMTQSPSSLSASVGDRVTITCKASQDVSSAVAWYQQKPGQAPRLLIYWASTRHTGVPSRFSGSGSGTEFTLTISSLQPDDFATYYCQEHFSTVLTFGQGTKVEIK

SEQ ID NO: 112 - protein, 107 aa, synthetic construct
  REGION 1..107: note = Synthetic sequence
DIQMTQSPSSLSASVGDRVTITCKASQDVSSAVAWYQQKPGQAPRLLIYWASTRHTGVPSRFSGSGSGTEFTLTISSLQPDDFATYYCQEHFSTWLTFGQGTKVEIK

SEQ ID NO: 113 - protein, 107 aa, synthetic construct
  REGION 1..107: note = Synthetic sequence
DIQMTQSPSSLSASVGDRVTITCKASQDVSSAVAWYQQKPGQAPRLLIYWASTRHTGVPSRFSGSGSGTEFTLTISSLQPDDFATYYCQEHFSTPGTFGQGTKVEIK

SEQ ID NO: 114 - protein, 107 aa, synthetic construct
  REGION 1..107: note = Synthetic sequence
DIQMTQSPSSLSASVGDRVTITCKASQDVSSAVAWYQQKPGQAPRLLIYWASTRHTGVPSRFSGSGSGTEFTLTISSLQPDDFATYYCQEHFSTPRTFGQGTKVEIK

SEQ ID NO: 115 - protein, 107 aa, synthetic construct
  REGION 1..107: note = Synthetic sequence
DIQMTQSPSSLSASVGDRVTITCKASQDVSSAVAWYQQKPGQAPRLLIYWASTRHTGVPSRFSGSGSGTEFTLTISSLQPDDFATYYCQEHFSTPLIFGQGTKVEIK

SEQ ID NO: 116 - protein, 107 aa, synthetic construct
  REGION 1..107: note = Synthetic sequence
DIQMTQSPSSLSASVGDRVTITCKASQDVSSAVAWYQQKPGQAPRLLIYWASTRHTGVPSRFSGSGSGTEFTLTISSLQPDDFATYYCQEHFSTPLRFGQGTKVEIK